European Patent Application EP 4 339 213 A1, published March 20, 2024. Title: ANTIGEN-BINDING MOLECULE. Applicant: JIANGSU HENGRUI PHARMACEUTICALS CO., LTD. SHANGHAI HENGRUI PHARMACEUTICAL CO., LTD. Application 22806844.1. The sequence listing filed with the application follows.

SEQUENCE LISTING (181 sequences)

SEQ ID NO: 1 - protein, 330 aa, Artificial Sequence [sequence omitted]

SEQ ID NO: 2 - protein, 330 aa, Artificial Sequence
  DOMAIN: Heavy chain constant region sequence of knob-IgG1
ASTKGPSVFPLAPSSKSTSGGTAALGCLVKDYFPEPVTVSWNSGALTSGVHTFPAVLQSSGLYSLSSVVTVPSSSLGTQTYICNVNHKPSNTKVDKKVEPKSCDKTHTCPPCPAPEAAGGPSVFLFPPKPKDTLMISRTPEVTCVVVDVSHEDPEVKFNWYVDGVEVHNAKTKPREEQYNSTYRVVSVLTVLHQDWLNGKEYKCKVSNKALPAPIEKTISKAKGQPREPQVYTLPPCREEMTKNQVSLWCLVKGFYPSDIAVEWESNGQPENNYKTTPPVLDSDGSFFLYSKLTVDKSRWQQGNVFSCSVMHEALHNHYTQKSLSLSPGK

SEQ ID NO: 3 - protein, 330 aa, Artificial Sequence
  DOMAIN: Heavy chain constant region sequence of hole-IgG1
ASTKGPSVFPLAPSSKSTSGGTAALGCLVKDYFPEPVTVSWNSGALTSGVHTFPAVLQSSGLYSLSSVVTVPSSSLGTQTYICNVNHKPSNTKVDKKVEPKSCDKTHTCPPCPAPEAAGGPSVFLFPPKPKDTLMISRTPEVTCVVVDVSHEDPEVKFNWYVDGVEVHNAKTKPREEQYNSTYRVVSVLTVLHQDWLNGKEYKCKVSNKALPAPIEKTISKAKGQPREPQVCTLPPSREEMTKNQVSLSCAVKGFYPSDIAVEWESNGQPENNYKTTPPVLDSDGSFFLVSKLTVDKSRWQQGNVFSCSVMHEALHNHYTQKSLSLSPGK

SEQ ID NO: 4 - protein, 107 aa, Artificial Sequence [sequence omitted]

SEQ ID NO: 5 - protein, 106 aa, Artificial Sequence
  DOMAIN: lambda light chain constant region sequence
GQPKAAPSVTLFPPSSEELQANKATLVCLISDFYPGAVTVAWKADSSPVKAGVETTTPSKQSNNKYAASSYLSLTPEQWKSHRSYSCQVTHEGSTVEKTVAPTECS

SEQ ID NO: 6 - protein, 119 aa, Artificial Sequence
  DOMAIN: VH sequence of F0 antibody
QVQLVQSGGGVVQPGTSLRLSCAASGFIFSSSAMHWVRQAPGKGLEWVAVISYDGSNKYYVDSVKGRFTISRDNSKNTLYLQMNSLRAEDTAVYYCARSARLYASFDYWGQGALVTVSS

SEQ ID NO: 7 - protein, 110 aa, Artificial Sequence
  DOMAIN: VL sequence of F0 antibody
DTVVTQEPSFSVSPGGTVTLTCGLSSGSVSTSHYPSWYQQTPGQAPRMLIYNTNTRSSGVPDRFSGSILGNKAALTITGAQADDESDYYCAIHVDRDIWVFGGGTKLTVL

SEQ ID NO: 8 - protein, 116 aa, Artificial Sequence
  DOMAIN: VH sequence of N0 antibody
DVQLVQSGGGLVQPGGSLRLSCAGSGFTSSLSWMSWLRQAPGKGLEWVANINQDGSEKNYVDSVKGRFTISRDNAQNSLYLQMSSLRAEDTAVYYCARGLWTFDSWGQGTLLTVSP

SEQ ID NO: 9 - protein, 108 aa, Artificial Sequence
  DOMAIN: VL sequence of N0 antibody
EIVLTQSPGTLSLSPGERATLSCRASQNINNRFLAWYQQRPGQAPRLLIYAASSRATGVPDRFSGSGSGTDFTLTISRLEAEDFAMYHCQQYGSFPRTFGQGTMVDIK

SEQ ID NO: 10 - protein, 120 aa, Artificial Sequence [sequence omitted]

SEQ ID NO: 11 - protein, 107 aa, Artificial Sequence [sequence omitted]

SEQ ID NO: 12 - protein, 121 aa, Artificial Sequence
  DOMAIN: VH sequence of V0 antibody
QVQLQQSAAELARPGASVKMSCKASGYSFTSYTIHWVKQRPGQGLEWIGYINPNSRNTDYNQKFKDETTLTADRSSSTAYMQLISLTSEDSAVYYCARYSGSTPYWYFDVWGAGTTVTVSS

SEQ ID NO: 13 - protein, 106 aa, Artificial Sequence
  DOMAIN: VL sequence of V0 antibody
QIVLTQSPAILSASPGEKVTMTCRASSSVSYMNWYQQKPGSSPKPWIYATSNLASGVPARFSVSVSGTSHSLTISRVEAEDAATYYCQQWSSNPLTFGAGTKLELK

SEQ ID NO: 14 - protein, 120 aa, Artificial Sequence
  DOMAIN: VH sequence of J0 antibody
EVQLVESGGGLVKPGGSLRLSCAASGFTFSDYWMHWVRQAPGKGLEWVGHIKSKTDAGTTDYAAPVKGRFTISRDDSKNTLYLQMNSLKTEDTAVYYCAREIYYYAFDSWGQGTLVTVSS

SEQ ID NO: 15 - protein, 107 aa, Artificial Sequence
  DOMAIN: VL sequence of J0 antibody
SYELTQPLSVSVALGQTARITCSGDNIGSKYVHWYQQKPGQAPVLVIYGDNERPSGIPERFSGSNSGNTATLTISRAQAGDEADYYCQAADWVDFYVFGGGTKLTVL

SEQ ID NO: 16 - protein, 118 aa, Artificial Sequence
  DOMAIN: VH sequence of H0 antibody
EVQLVESGGGLVQPGGSLRLSCAASGFTFSHYYMAWVRQAPGKGLEWVTSISYEGDITYYGDSVKGRFTISRDNSKNTLYLQMNSLRAEDTATYYCASQTLRESFDYWGQGTLVTVSS

SEQ ID NO: 17 - protein, 107 aa, Artificial Sequence
  DOMAIN: VL sequence of H0 antibody
DIQMTQSPSSVSASVGDRVTITCRASQDIANYLSWYQQKPGKSPKLLIYGTSNLEVGVPSRFSGSRSGTDFTLTISSLQPEDFATYYCLQDKEFPRTFGGGTKVEIK

SEQ ID NO: 18 - protein, 116 aa, Artificial Sequence [sequence omitted]

SEQ ID NO: 19 - protein, 107 aa, Artificial Sequence [sequence omitted]

SEQ ID NO: 20 - protein, 123 aa, Artificial Sequence
  DOMAIN: VH sequence of B0 antibody
QVQLQQSGAEVKKPGSSVRVSCKASGGTFNNNAINWVRQAPGQGLEWMGGIIPMFGTAKYSQNFQGRVAITADESTGTASMELSSLRSEDTAVYYCARSRDLLLFPHHALSPWGRGTMVTVSS

SEQ ID NO: 21 - protein, 108 aa, Artificial Sequence
  DOMAIN: VL sequence of B0 antibody
SSELTQDPAVSVALGQTVRVTCQGDSLRSYYASWYQQKPGQAPVLVIYGKNNRPSGIPDRFSGSSSGNTASLTITGAQAEDEADYYCSSRDSSGNHWVFGGGTELTVL

SEQ ID NO: 22 - protein, 119 aa, Artificial Sequence
  DOMAIN: VH sequence of U0 antibody
EVQLVQSGAEVKKPGESLKISCKGSGYSFTTYWLGWVRQMPGKGLDWIGIMSPVDSDIRYSPSFQGQVTMSVDKSITTAYLQWNSLKASDTAMYYCARRRPGQGYFDFWGQGTLVTVSS

SEQ ID NO: 23 - protein, 107 aa, Artificial Sequence
  DOMAIN: VL sequence of U0 antibody
DIQMTQSPSSLSASVGDRVTITCRASQGISSWLAWYQQKPEKAPKSLIYAASSLQSGVPSRFSGSGSGTDFTLTISSLQPEDFATYYCQQYNIYPYTFGQGTKLEIK

SEQ ID NO: 24 - protein, 122 aa, Artificial Sequence
  DOMAIN: VH sequence of D0 antibody
EVQLLESGGGLVQPGGSLRLSCAASGFTFSSYAMSWVRQAPGKGLEWVSGITGSGGSTYYADSVKGRFTISRDNSKNTLYLQMNSLRAEDTAVYYCAKDPGTTVIMSWFDPWGQGTLVTVSS

SEQ ID NO: 25 - protein, 108 aa, Artificial Sequence
  DOMAIN: VL sequence of D0 antibody
EIVLTQSPGTLSLSPGERATLSCRASQSVRGRYLAWYQQKPGQAPRLLIYGASSRATGIPDRFSGSGSGTDFTLTISRLEPEDFAVFYCQQYGSSPRTFGQGTKVEIK

SEQ ID NO: 26 - protein, 121 aa, Artificial Sequence [sequence omitted]

SEQ ID NO: 27 - protein, 107 aa, Artificial Sequence [sequence omitted]

SEQ ID NO: 28 - protein, 117 aa, Artificial Sequence
  DOMAIN: VH sequence of C0 antibody
EVQLVQSGAEVKKPGASVKVSCKASGYTFTDYHMNWVRQAPGQRLEWMGDINPDIGGTSYNQNFKGRVTITRDTSASTAYMELSSLRSEDTAVYYCARWDFDSFANWGQGTLVTVSS

SEQ ID NO: 29 - protein, 111 aa, Artificial Sequence
  DOMAIN: VL sequence of C0 antibody
DIVMTQSPDSLAVSLGERATINCRASESVSIIGTNLIHWYQQKPGQPPKLLIYHASNLETGVPDRFSGSGSGTDFTLTISSLQAEDVAVYYCLQSRKIPYTFGGGTKVEIK

SEQ ID NO: 30 - protein, 104 aa, Artificial Sequence
  DOMAIN: IL6Ra.0 chain sequence
GILQPDPPANITVTAVARNPRWLSVTWQDPHSWNSSFYRLRFELRYRAERSKTFTTWMVKDLQHHCVIHDAWSGLRHVVQLRAQEEFGQGEWSEWSPEAMGTPW

SEQ ID NO: 31 - protein, 108 aa, Artificial Sequence
  DOMAIN: IL6Rb.0 chain sequence
FDPVYKVKPNPPHNLSVINSEELSSILKLTWTNPSIKSVIILKYNIQYRTKDASTWSQIPPEDTASTRSSFTVQDLKPFTEYVFRIRCMKEDGKGYWSDWSEEASGIT

SEQ ID NO: 32 - protein, 98 aa, Artificial Sequence
  DOMAIN: T.0 chain sequence
GIPPKIEALPSDISIDEGKVLTVACAFTGEPTPEVTWSCGGRKIHSQEQGRFHIENTDDLTTLIIMDVQKQDGGLYTLSLGNEFGSDSATVNIHIRSI

SEQ ID NO: 33 - protein, 97 aa, Artificial Sequence
  DOMAIN: O.0 chain sequence
SGAPRFLTRPKAFVVSVGKDATLSCQIVGNPTPQVSWEKDQQPVAAGARFRLAQDGDLYRLTILDLALGDSGQYVCRARNAIGEAFAAVGLQVDAEA

SEQ ID NO: 34 - protein, 98 aa, Artificial Sequence
  DOMAIN: OL.0 chain sequence
QGSPPCFLRFPRPVRVVSGAEAELKCVVLGEPPPVVVWEKGGQQLAASERLSFPADGAEHGLLLTAALPTDAGVYVCRARNAAGEAYAAAAVTVLEPP

SEQ ID NO: 35 - protein, 98 aa, Artificial Sequence
  DOMAIN: T.1 chain sequence
GIPPKIECLPSDISIDEGKVLTVASAFTGEPTPEVTWSTGGRKIHSQEQGRFHIENTDDLTTLIIMDVQKQDGGLYTLSLGNEFGSDSATVNIHIRSI

SEQ ID NO: 36 - protein, 98 aa, Artificial Sequence
  DOMAIN: T.2 chain sequence
GIPPKIEALPSDISIDEGKCLTVASAFTGEPTPEVTWSTGGRKIHSQEQGRFHIENTDDLTTLIIMDVQKQDGGLYTLSLGNEFGSDSATVNIHIRSI

SEQ ID NO: 37 - protein, 98 aa, Artificial Sequence
  DOMAIN: T.3 chain sequence
GIPPKIEALPSDISIDEGKVLTVASCFTGEPTPEVTWSTGGRKIHSQEQGRFHIENTDDLTTLIIMDVQKQDGGLYTLSLGNEFGSDSATVNIHIRSI

SEQ ID NO: 38 - protein, 98 aa, Artificial Sequence
  DOMAIN: T.4 chain sequence
GIPPKIEALPSDISIDEGKVLCVASAFTGEPTPEVTWSTGGRKIHSQEQGRFHIENTDDLTTLIIMDVQKQDGGLYTLSLGNEFGSDSATVNIHIRSI

SEQ ID NO: 39 - protein, 103 aa, Artificial Sequence
  DOMAIN: T.5 chain sequence
KAGIRGIPPKIECLPSDISIDEGKVLTVASAFTGEPTPEVTWSTGGRKIHSQEQGRFHIENTDDLTTLIIMDVQKQDGGLYTLSLGNEFGSDSATVNIHIRSI

SEQ ID NO: 40 - protein, 103 aa, Artificial Sequence
  DOMAIN: T.1-L1 chain sequence
GGGGSGIPPKIECLPSDISIDEGKVLTVASAFTGEPTPEVTWSTGGRKIHSQEQGRFHIENTDDLTTLIIMDVQKQDGGLYTLSLGNEFGSDSATVNIHIRSI

SEQ ID NO: 41 - protein, 108 aa, Artificial Sequence
  DOMAIN: T.1-L2 chain sequence
GGGGSGGGGSGIPPKIECLPSDISIDEGKVLTVASAFTGEPTPEVTWSTGGRKIHSQEQGRFHIENTDDLTTLIIMDVQKQDGGLYTLSLGNEFGSDSATVNIHIRSI

SEQ ID NO: 42 - protein, 97 aa, Artificial Sequence
  DOMAIN: O.1 chain sequence
SGAPRFLTRPKAFVVSVGKDATLSCQIVGNPTPQVSWEKDQQPVAAGARFRLAQDGDLYRLTILDLALGDSGQYVCRARNAIGEAFACVGLQVDAEA

SEQ ID NO: 43 - protein, 97 aa, Artificial Sequence
  DOMAIN: O.2 chain sequence
SGCPRFLTRPKAFVVSVGKDATLSCQIVGNPTPQVSWEKDQQPVAAGARFRLAQDGDLYRLTILDLALGDSGQYVCRARNAIGEAFAAVGLQVDAEA

SEQ ID NO: 44 - protein, 97 aa, Artificial Sequence
  DOMAIN: O.3 chain sequence
SGAPRFLTCPKAFVVSVGKDATLSCQIVGNPTPQVSWEKDQQPVAAGARFRLAQDGDLYRLTILDLALGDSGQYVCRARNAIGEAFAAVGLQVDAEA

SEQ ID NO: 45 - protein, 97 aa, Artificial Sequence
  DOMAIN: O.4 chain sequence
SGAPRFLTRPKAFVVSVGKDATLSSQIVGNPTPQVSWEKDQQPVAAGARFRLAQDGDLYRLTILDLALGDSGQYVSRARNAIGEAFACVGLQVDAEA

SEQ ID NO: 46 - protein, 97 aa, Artificial Sequence
  DOMAIN: O.5 chain sequence
SGCPRFLTRPKAFVVSVGKDATLSSQIVGNPTPQVSWEKDQQPVAAGARFRLAQDGDLYRLTILDLALGDSGQYVSRARNAIGEAFAAVGLQVDAEA

SEQ ID NO: 47 - protein, 97 aa, Artificial Sequence
  DOMAIN: O.6 chain sequence
SGAPRFLTCPKAFVVSVGKDATLSSQIVGNPTPQVSWEKDQQPVAAGARFRLAQDGDLYRLTILDLALGDSGQYVSRARNAIGEAFAAVGLQVDAEA

SEQ ID NO: 48 - protein, 97 aa, Artificial Sequence
  DOMAIN: O.7 chain sequence
SGAPRFKTRPKAFVVSVGKDATLSSQIVGNPTPQVSWEKDQQPVAAGARFRLAQDGDLYRLKILDLALGDSGQYVSRARNAIGEAFACVGLQVDAEA

SEQ ID NO: 49 - protein, 97 aa, Artificial Sequence
  DOMAIN: O.8 chain sequence
SGAPRFKTRPKAFVVSVGKDATLSSQIVGNPTPQVSWEKDQQPVAAGARFRLAQDGDLYRLHILDLALGDSGQYVSRARNAIGEAFACVGLQVDAEA

SEQ ID NO: 50 - protein, 97 aa, Artificial Sequence
  DOMAIN: O.9 chain sequence
SGAPRFLTRPLAFVVSVGKDATLSSQIVGNPTPQVSWEKDQQPVAAGARFRLAQDGDLYRLKILDLALGDSGQYVSRARNAIGEAFACVGLQVDAEA

SEQ ID NO: 51 - protein, 97 aa, Artificial Sequence
  DOMAIN: O.10 chain sequence
SGAPRFLTRPLAFVVSVGKDATLSSQIVGNPTPQVSWEKDQQPVAAGARFRLAQDGDLYRLHILDLALGDSGQYVSRARNAIGEAFACVGLQVDAEA

SEQ ID NO: 52 - protein, 102 aa, Artificial Sequence
  DOMAIN: O.11 chain sequence
DQPQFSGAPRFLTRPKAFVVSVGKDATLSSQIVGNPTPQVSWEKDQQPVAAGARFRLAQDGDLYRLTILDLALGDSGQYVSRARNAIGEAFACVGLQVDAEA

SEQ ID NO: 53 - protein, 102 aa, Artificial Sequence
  DOMAIN: O.12 chain sequence
DQPQFSGAPRFKTRPKAFVVSVGKDATLSSQIVGNPTPQVSWEKDQQPVAAGARFRLAQDGDLYRLKILDLALGDSGQYVSRARNAIGEAFACVGLQVDAEA

SEQ ID NO: 54 - protein, 102 aa, Artificial Sequence
  DOMAIN: O.13 chain sequence
DQPQFSGAPRFKTRPKAFVVSVGKDATLSSQIVGNPTPQVSWEKDQQPVAAGARFRLAQDGDLYRLHILDLALGDSGQYVSRARNAIGEAFACVGLQVDAEA

SEQ ID NO: 55 - protein, 102 aa, Artificial Sequence
  DOMAIN: O.14 chain sequence
DQPQFSGAPRFRTRPKAFVVSVGKDATLSSQIVGNPTPQVSWEKDQQPVAAGARFRLAQDGDLYRLKILDLALGDSGQYVSRARNAIGEAFACVGLQVDAEA

SEQ ID NO: 56 - protein, 102 aa, Artificial Sequence
  DOMAIN: O.15 chain sequence
DQPQFSGAPRFRTRPKAFVVSVGKDATLSSQIVGNPTPQVSWEKDQQPVAAGARFRLAQDGDLYRLHILDLALGDSGQYVSRARNAIGEAFACVGLQVDAEA

SEQ ID NO: 57 - protein, 102 aa, Artificial Sequence
  DOMAIN: O.4-L1 chain sequence
GGGGSSGAPRFLTRPKAFVVSVGKDATLSSQIVGNPTPQVSWEKDQQPVAAGARFRLAQDGDLYRLTILDLALGDSGQYVSRARNAIGEAFACVGLQVDAEA

SEQ ID NO: 58 - protein, 107 aa, Artificial Sequence
  DOMAIN: O.4-L2 chain sequence
GGGGSGGGGSSGAPRFLTRPKAFVVSVGKDATLSSQIVGNPTPQVSWEKDQQPVAAGARFRLAQDGDLYRLTILDLALGDSGQYVSRARNAIGEAFACVGLQVDAEA

SEQ ID NO: 59 - protein, 98 aa, Artificial Sequence
  DOMAIN: OL.1 chain sequence
QGSPPEFLRFPRPVRVVSGAEAELKCVVLGEPPPVVVWEKGGQQLAASERLSFPADGAEHGLLLTAALPTDAGCYVCRARNAAGEAYAAAAVTVLEPP

SEQ ID NO: 60 - protein, 98 aa, Artificial Sequence
  DOMAIN: OL.2 chain sequence
QGSPPEFLRFPRPVRVVSGAEAELKCVVLGEPPPVVVWEKGGQQLAASERLSFPADGAEHGLLLTAALPTDAGVYVCRARNAACEAYAAAAVTVLEPP

SEQ ID NO: 61 - protein, 98 aa, Artificial Sequence
  DOMAIN: OL.3 chain sequence
QGSPPEFLRFPRPVRVVSGAEAELKCVVLGEPPPVVVWEKGGQQLAASERLSFPADGAEHGLLLTAALPTDAGVYVCRARNAAGECYAAAAVTVLEPP

SEQ ID NO: 62 - protein, 98 aa, Artificial Sequence
  DOMAIN: OL.4 chain sequence
QGSPPEFLRFPRPVRVVSGAEAELKSVVLGEPPPVVVWEKGGQQLAASERLSFPADGAEHGLLLTAALPTDAGCYVSRARNAAGEAYAAAAVTVLEPP

SEQ ID NO: 63 - protein, 98 aa, Artificial Sequence
  DOMAIN: OL.5 chain sequence
QGSPPEFLRFPRPVRVVSGAEAELKSVVLGEPPPVVVWEKGGQQLAASERLSFPADGAEHGLLLTAALPTDAGVYVSRARNAACEAYAAAAVTVLEPP

SEQ ID NO: 64 - protein, 98 aa, Artificial Sequence
  DOMAIN: OL.6 chain sequence
QGSPPEFLRFPRPVRVVSGAEAELKSVVLGEPPPVVVWEKGGQQLAASERLSFPADGAEHGLLLTAALPTDAGVYVSRARNAAGECYAAAAVTVLEPP

SEQ ID NO: 65 - protein, 98 aa, Artificial Sequence
  DOMAIN: T.7 chain sequence
GIPPKIECLPSDISIDEGKVLTVASAFTGEPTPEVTWSTGGRKIHSQEQGRFHIENTDDLTTLIISDVQKQDGGLYSLSLGNEFGSDSATVNIHIRSI

SEQ ID NO: 66 - protein, 98 aa, Artificial Sequence
  DOMAIN: T.8 chain sequence
GIPPKIECLPSDISIDEGKVLTVASAFTGEPTPEVTWSTGGRKIHSQEQGRFHIENTDDLTTLIIKDVQRQDGGLYTLTLRNEFGSDSATVNIHIRSI

SEQ ID NO: 67 - protein, 98 aa, Artificial Sequence
  DOMAIN: T.9 chain sequence
GIWPKIECLPIDLSIDEGKVLMVASAFTGEPTPEVTWSTGGRKIHSQEQGRFHIENTDDLTTLIIMDVQKQDGGLYTLSLGMEFGSDSATVNIHIRSI

SEQ ID NO: 68 - protein, 98 aa, Artificial Sequence
  DOMAIN: T.10 chain sequence
GIPPKIECLPIDISIDEGKVLTVASAFTGEPTPEVTWSTGGRKIHSQEQGRFHIENTDDLTTLIIKDVQKQDGGLYTLTLRNEFGSDSATVNIHIRSI

SEQ ID NO: 69 - protein, 98 aa, Artificial Sequence
  DOMAIN: T.11 chain sequence
GIPPKIECLPSDISIDEGKVLTVASAFTGEPTPEVTWSTSGKKISSEEGGRFHIESTEDLTTLIIMDVQKQDGGVYTLSLGNDLGSDSATVNIHIRSI

SEQ ID NO: 70 - protein, 98 aa, Artificial Sequence
  DOMAIN: T.12 chain sequence
GIPPKIECLPSDISIDEGKVLTVASAFTGEPTPEVTWSTGGRKIHSEEGGRFHIESTEDLTTLIIMDVQKQDGGVYTLSLGNEFGSDSATVNIHIRSI

SEQ ID NO: 71 - protein, 98 aa, Artificial Sequence
  DOMAIN: T.13 chain sequence
GIPPKIECLPSDISIDEGKVLTVASAFTGEPTPEVTWSTGGRKIHSQEQGRFHIESTEDLTTLIIMDVQKQDGGVYTLSLGNEFGSDSATVNIHIRSI

SEQ ID NO: 72 - protein, 98 aa, Artificial Sequence
  DOMAIN: T.14 chain sequence
GIPPKIECLPSDISIDEGKVLTVASAFTGEPTPEVTWSTGGRKIHSQEQGRFHIESTEDLTTLIISDVQKQDGGLYSLSLGNEFGSDSATVNIHIRSI

SEQ ID NO: 73 - protein, 103 aa, Artificial Sequence
  DOMAIN: T.10-L1 sequence
GGGGSGIPPKIECLPIDISIDEGKVLTVASAFTGEPTPEVTWSTGGRKIHSQEQGRFHIENTDDLTTLIIKDVQKQDGGLYTLTLRNEFGSDSATVNIHIRSI

SEQ ID NO: 74 - protein, 103 aa, Artificial Sequence
  DOMAIN: T.15 chain sequence
KAGIRGIPPKIECLPSDISIDEGKVLTVASAFTGEPTPEVTWSTGGRKIHSQEQGRFHIESTEDLTTLIISDVQKQDGGLYSLSLGNEFGSDSATVNIHIRSI

SEQ ID NO: 75 - protein, 108 aa, Artificial Sequence
  DOMAIN: T.15-L1 chain sequence
GGGGSKAGIRGIPPKIECLPSDISIDEGKVLTVASAFTGEPTPEVTWSTGGRKIHSQEQGRFHIESTEDLTTLIISDVQKQDGGLYSLSLGNEFGSDSATVNIHIRSI

SEQ ID NO: 76 - protein, 103 aa, Artificial Sequence
  DOMAIN: T.14-L1 chain sequence
GGGGSGIPPKIECLPSDISIDEGKVLTVASAFTGEPTPEVTWSTGGRKIHSQEQGRFHIESTEDLTTLIISDVQKQDGGLYSLSLGNEFGSDSATVNIHIRSI

SEQ ID NO: 77 - protein, 97 aa, Artificial Sequence
  DOMAIN: O.17 chain sequence
SGAPRFLTRPKSYTVSVGKDASLSSQIVGNPTPQVSWEKDQQPVAAGARFRLAQDGDLYRLKILDLALGDSGQYVSRARNAIGEAFACVGLQVDAEA

SEQ ID NO: 78 - protein, 97 aa, Artificial Sequence
  DOMAIN: O.18 chain sequence
SEAPRFLTRPLAFVVSEGKDATLSSQIVGDPPPEVTWEKDQQPITAGARFRLAQDGDVYRLEILDLQLSDSGQYVSRARNAIGEAFACVGLQVDAEG

SEQ ID NO: 79 - protein, 97 aa, Artificial Sequence
  DOMAIN: O.19 chain sequence
SGAPRFLTRPLAFVVSVGKLAMLSSQIVGNPTPQVSWEKDQQPVAAGARFRLLQDGDLYRLKILDLALGDSGQYVSRARNAIGEAFACVGLQVDAEA

SEQ ID NO: 80 - protein, 97 aa, Artificial Sequence
  DOMAIN: O.20 chain sequence
SGAPRFLTRPLAFVVSVGKDATLSSQIVGNPTPQVSWEKDKQPVTAGARFRLAQDGDLYRLKILDLQLSDSGQYVSRARNAIGEAFACLGLQVDAEA

SEQ ID NO: 81 - protein, 97 aa, Artificial Sequence
  DOMAIN: O.21 chain sequence
SGAPRFLTRPLAFVVSVGKDATLSSQIVGNPTPQVSWEKDQLPVTAGARFRLAQDGDLYRLKILDLTLSDSGQYVSRARNAIGEAFACVGLEVGAEA

SEQ ID NO: 82 - protein, 97 aa, Artificial Sequence
  DOMAIN: O.22 chain sequence
SGAPRFLTRPLSYVVSVGKDASLSSQIVGNPTPQVSWEKDQLPVTAGARFRLAQDGDLYRLKILDLQLSDSGQYVSRARNAIGEAFACVGLEVGAEA

SEQ ID NO: 83 - protein, 102 aa, Artificial Sequence
  DOMAIN: O.20-L1 chain sequence
GGGGSSGAPRFLTRPLAFVVSVGKDATLSSQIVGNPTPQVSWEKDKQPVTAGARFRLAQDGDLYRLKILDLQLSDSGQYVSRARNAIGEAFACLGLQVDAEA

SEQ ID NO: 84 - protein, 102 aa, Artificial Sequence
  DOMAIN: O.22-L1 chain sequence
GGGGSSGAPRFLTRPLSYVVSVGKDASLSSQIVGNPTPQVSWEKDQLPVTAGARFRLAQDGDLYRLKILDLQLSDSGQYVSRARNAIGEAFACVGLEVGAEA

SEQ ID NO: 85 - protein, 102 aa, Artificial Sequence
  DOMAIN: O.23 chain sequence
DQPQFSGAPRFLTRPLSYVVSVGKDASLSSQIVGNPTPQVSWEKDQLPVTAGARFRLAQDGDLYRLKILDLQLSDSGQYVSRARNAIGEAFACVGLEVGAEA

SEQ ID NO: 86 - protein, 107 aa, Artificial Sequence
  DOMAIN: O.23-L1 sequence
GGGGSDQPQFSGAPRFLTRPLSYVVSVGKDASLSSQIVGNPTPQVSWEKDQLPVTAGARFRLAQDGDLYRLKILDLQLSDSGQYVSRARNAIGEAFACVGLEVGAEA

SEQ ID NO: 87 - protein, 452 aa, Artificial Sequence
  CHAIN: Sequence of DI-1 chain 1 (DI-1-H1)
EVQLLESGGGLVQPGGSLRLSCAASGFTFSSYAMSWVRQAPGKGLEWVSGITGSGGSTYYADSVKGRFTISRDNSKNTLYLQMNSLRAEDTAVYYCAKDPGTTVIMSWFDPWGQGTLVTVSSASTKGPSVFPLAPSSKSTSGGTAALGCLVKDYFPEPVTVSWNSGALTSGVHTFPAVLQSSGLYSLSSVVTVPSSSLGTQTYICNVNHKPSNTKVDKKVEPKSCDKTHTCPPCPAPEAAGGPSVFLFPPKPKDTLMISRTPEVTCVVVDVSHEDPEVKFNWYVDGVEVHNAKTKPREEQYNSTYRVVSVLTVLHQDWLNGKEYKCKVSNKALPAPIEKTISKAKGQPREPQVYTLPPCREEMTKNQVSLWCLVKGFYPSDIAVEWESNGQPENNYKTTPPVLDSDGSFFLYSKLTVDKSRWQQGNVFSCSVMHEALHNHYTQKSLSLSPGK

SEQ ID NO: 88 - protein, 215 aa, Artificial Sequence
  CHAIN: Sequence of DI-1 chain 2 (DI-1-L1)
EIVLTQSPGTLSLSPGERATLSCRASQSVRGRYLAWYQQKPGQAPRLLIYGASSRATGIPDRFSGSGSGTDFTLTISRLEPEDFAVFYCQQYGSSPRTFGQGTKVEIKRTVAAPSVFIFPPSDEQLKSGTASVVCLLNNFYPREAKVQWKVDNALQSGNSQESVTEQDSKDSTYSLSSTLTLSKADYEKHKVYACEVTHQGLSSPVTKSFNRGEC

SEQ ID NO: 89 - protein, 451 aa, Artificial Sequence
  CHAIN: Sequence of DI-1 chain 3 (DI-1-H2)
QVQLQESGPGLVKPSETLSLTCTVSGFSLIGYDLNWIRQPPGKGLEWIGIIWGDGTTDYNSAVKSRVTISKDTSKNQFSLKLSSVTAADTAVYYCARGGYWYATSYYFDYWGQGTLVTVSSGGGGSGIPPKIECLPIDISIDEGKVLTVASAFTGEPTPEVTWSTGGRKIHSQEQGRFHIENTDDLTTLIIKDVQKQDGGLYTLTLRNEFGSDSATVNIHIRSIDKTHTCPPCPAPEAAGGPSVFLFPPKPKDTLMISRTPEVTCVVVDVSHEDPEVKFNWYVDGVEVHNAKTKPREEQYNSTYRVVSVLTVLHQDWLNGKEYKCKVSNKALPAPIEKTISKAKGQPREPQVCTLPPSREEMTKNQVSLSCAVKGFYPSDIAVEWESNGQPENNYKTTPPVLDSDGSFFLVSKLTVDKSRWQQGNVFSCSVMHEALHNHYTQKSLSLSPGK

SEQ ID NO: 90 - protein, 209 aa, Artificial Sequence
  CHAIN: Sequence of DI-1 chain 4 (DI-1-L2)
DIQMTQSPSSLSASVGDRVTITCRASQSISNNLNWYQQKPGKAPKLLIYYTSRFHSGVPSRFSGSGSGTDFTFTISSLQPEDIATYYCQQEHTLPYTFGQGTKLEIKGGGGSSGAPRFLTRPLAFVVSVGKDATLSSQIVGNPTPQVSWEKDKQPVTAGARFRLAQDGDLYRLKILDLQLSDSGQYVSRARNAIGEAFACLGLQVDAEA

SEQ ID NO: 91 - protein, 453 aa, Artificial Sequence
  CHAIN: Sequence of BU1 chain 1 (BU1-H1)
QVQLQQSGAEVKKPGSSVRVSCKASGGTFNNNAINWVRQAPGQGLEWMGGIIPMFGTAKYSQNFQGRVAITADESTGTASMELSSLRSEDTAVYYCARSRDLLLFPHHALSPWGRGTMVTVSSASTKGPSVFPLAPSSKSTSGGTAALGCLVKDYFPEPVTVSWNSGALTSGVHTFPAVLQSSGLYSLSSVVTVPSSSLGTQTYICNVNHKPSNTKVDKKVEPKSCDKTHTCPPCPAPEAAGGPSVFLFPPKPKDTLMISRTPEVTCVVVDVSHEDPEVKFNWYVDGVEVHNAKTKPREEQYNSTYRVVSVLTVLHQDWLNGKEYKCKVSNKALPAPIEKTISKAKGQPREPQVYTLPPCREEMTKNQVSLWCLVKGFYPSDIAVEWESNGQPENNYKTTPPVLDSDGSFFLYSKLTVDKSRWQQGNVFSCSVMHEALHNHYTQKSLSLSPGK

SEQ ID NO: 92 - protein, 214 aa, Artificial Sequence
  CHAIN: Sequence of BU1 chain 2 (BU1-L1)
SSELTQDPAVSVALGQTVRVTCQGDSLRSYYASWYQQKPGQAPVLVIYGKNNRPSGIPDRFSGSSSGNTASLTITGAQAEDEADYYCSSRDSSGNHWVFGGGTELTVLGQPKAAPSVTLFPPSSEELQANKATLVCLISDFYPGAVTVAWKADSSPVKAGVETTTPSKQSNNKYAASSYLSLTPEQWKSHRSYSCQVTHEGSTVEKTVAPTECS

SEQ ID NO: 93 - protein, 449 aa, Artificial Sequence
  CHAIN: Sequence of BU1 chain 3 (BU1-H2)
EVQLVQSGAEVKKPGESLKISCKGSGYSFTTYWLGWVRQMPGKGLDWIGIMSPVDSDIRYSPSFQGQVTMSVDKSITTAYLQWNSLKASDTAMYYCARRRPGQGYFDFWGQGTLVTVSSGGGGSGIPPKIECLPSDISIDEGKVLTVASAFTGEPTPEVTWSTGGRKIHSQEQGRFHIESTEDLTTLIISDVQKQDGGLYSLSLGNEFGSDSATVNIHIRSIDKTHTCPPCPAPEAAGGPSVFLFPPKPKDTLMISRTPEVTCVVVDVSHEDPEVKFNWYVDGVEVHNAKTKPREEQYNSTYRVVSVLTVLHQDWLNGKEYKCKVSNKALPAPIEKTISKAKGQPREPQVCTLPPSREEMTKNQVSLSCAVKGFYPSDIAVEWESNGQPENNYKTTPPVLDSDGSFFLVSKLTVDKSRWQQGNVFSCSVMHEALHNHYTQKSLSLSPGK

SEQ ID NO: 94 - protein, 209 aa, Artificial Sequence
  CHAIN: Sequence of BU1 chain 4 (BU1-L2)
DIQMTQSPSSLSASVGDRVTITCRASQGISSWLAWYQQKPEKAPKSLIYAASSLQSGVPSRFSGSGSGTDFTLTISSLQPEDFATYYCQQYNIYPYTFGQGTKLEIKGGGGSSGAPRFLTRPLSYVVSVGKDASLSSQIVGNPTPQVSWEKDQLPVTAGARFRLAQDGDLYRLKILDLQLSDSGQYVSRARNAIGEAFACVGLEVGAEA

SEQ ID NO: 95 - protein, 449 aa, Artificial Sequence
  CHAIN: Sequence of BU2 chain 1 (BU2-H1)/BU4 chain 1 (BU4-H1)/BU5 chain 3 (BU5-H2)
EVQLVQSGAEVKKPGESLKISCKGSGYSFTTYWLGWVRQMPGKGLDWIGIMSPVDSDIRYSPSFQGQVTMSVDKSITTAYLQWNSLKASDTAMYYCARRRPGQGYFDFWGQGTLVTVSSASTKGPSVFPLAPSSKSTSGGTAALGCLVKDYFPEPVTVSWNSGALTSGVHTFPAVLQSSGLYSLSSVVTVPSSSLGTQTYICNVNHKPSNTKVDKKVEPKSCDKTHTCPPCPAPEAAGGPSVFLFPPKPKDTLMISRTPEVTCVVVDVSHEDPEVKFNWYVDGVEVHNAKTKPREEQYNSTYRVVSVLTVLHQDWLNGKEYKCKVSNKALPAPIEKTISKAKGQPREPQVYTLPPCREEMTKNQVSLWCLVKGFYPSDIAVEWESNGQPENNYKTTPPVLDSDGSFFLYSKLTVDKSRWQQGNVFSCSVMHEALHNHYTQKSLSLSPGK

SEQ ID NO: 96 - protein, 214 aa, Artificial Sequence
  CHAIN: Sequence of BU2 chain 2 (BU2-L1)/BU3 chain 4 (BU3-L2)/BU4 chain 2 (BU4-L1)/BU5 chain 4 (BU5-L2)
DIQMTQSPSSLSASVGDRVTITCRASQGISSWLAWYQQKPEKAPKSLIYAASSLQSGVPSRFSGSGSGTDFTLTISSLQPEDFATYYCQQYNIYPYTFGQGTKLEIKRTVAAPSVFIFPPSDEQLKSGTASVVCLLNNFYPREAKVQWKVDNALQSGNSQESVTEQDSKDSTYSLSSTLTLSKADYEKHKVYACEVTHQGLSSPVTKSFNRGEC

SEQ ID NO: 97 - protein, 453 aa, Artificial Sequence
  CHAIN: Sequence of BU2 chain 3 (BU2-H2)
QVQLQQSGAEVKKPGSSVRVSCKASGGTFNNNAINWVRQAPGQGLEWMGGIIPMFGTAKYSQNFQGRVAITADESTGTASMELSSLRSEDTAVYYCARSRDLLLFPHHALSPWGRGTMVTVSSGGGGSGIPPKIECLPSDISIDEGKVLTVASAFTGEPTPEVTWSTGGRKIHSQEQGRFHIESTEDLTTLIISDVQKQDGGLYSLSLGNEFGSDSATVNIHIRSIDKTHTCPPCPAPEAAGGPSVFLFPPKPKDTLMISRTPEVTCVVVDVSHEDPEVKFNWYVDGVEVHNAKTKPREEQYNSTYRVVSVLTVLHQDWLNGKEYKCKVSNKALPAPIEKTISKAKGQPREPQVCTLPPSREEMTKNQVSLSCAVKGFYPSDIAVEWESNGQPENNYKTTPPVLDSDGSFFLVSKLTVDKSRWQQGNVFSCSVMHEALHNHYTQKSLSLSPGK

SEQ ID NO: 98 - protein, 215 aa, Artificial Sequence
  CHAIN: Sequence of BU2 chain 4 (BU2-L2)
SSELTQDPAVSVALGQTVRVTCQGDSLRSYYASWYQQKPGQAPVLVIYGKNNRPSGIPDRFSGSSSGNTASLTITGAQAEDEADYYCSSRDSSGNHWVFGGGTELTVLGGGGSDQPQFSGAPRFLTRPLSYVVSVGKDASLSSQIVGNPTPQVSWEKDQLPVTAGARFRLAQDGDLYRLKILDLQLSDSGQYVSRARNAIGEAFACVGLEVGAEA

SEQ ID NO: 99 - protein, 453 aa, Artificial Sequence
  CHAIN: Sequence of BU3 chain 1 (BU3-H1)
QVQLQQSGAEVKKPGSSVRVSCKASGGTFNNNAINWVRQAPGQGLEWMGGIIPMFGTAKYSQNFQGRVAITADESTGTASMELSSLRSEDTAVYYCARSRDLLLFPHHALSPWGRGTMVTVSSGGGGSGIPPKIECLPSDISIDEGKVLTVASAFTGEPTPEVTWSTGGRKIHSQEQGRFHIESTEDLTTLIISDVQKQDGGLYSLSLGNEFGSDSATVNIHIRSIDKTHTCPPCPAPEAAGGPSVFLFPPKPKDTLMISRTPEVTCVVVDVSHEDPEVKFNWYVDGVEVHNAKTKPREEQYNSTYRVVSVLTVLHQDWLNGKEYKCKVSNKALPAPIEKTISKAKGQPREPQVYTLPPCREEMTKNQVSLWCLVKGFYPSDIAVEWESNGQPENNYKTTPPVLDSDGSFFLYSKLTVDKSRWQQGNVFSCSVMHEALHNHYTQKSLSLSPGK

SEQ ID NO: 100 - protein, 215 aa, Artificial Sequence; identical to SEQ ID NO: 98
  CHAIN: Sequence of BU3 chain 2 (BU3-L1)/BU4 chain 4 (BU4-L2)

SEQ ID NO: 101 - protein, 449 aa, Artificial Sequence
  CHAIN: Sequence of BU3 chain 3 (BU3-H2)
EVQLVQSGAEVKKPGESLKISCKGSGYSFTTYWLGWVRQMPGKGLDWIGIMSPVDSDIRYSPSFQGQVTMSVDKSITTAYLQWNSLKASDTAMYYCARRRPGQGYFDFWGQGTLVTVSSASTKGPSVFPLAPSSKSTSGGTAALGCLVKDYFPEPVTVSWNSGALTSGVHTFPAVLQSSGLYSLSSVVTVPSSSLGTQTYICNVNHKPSNTKVDKKVEPKSCDKTHTCPPCPAPEAAGGPSVFLFPPKPKDTLMISRTPEVTCVVVDVSHEDPEVKFNWYVDGVEVHNAKTKPREEQYNSTYRVVSVLTVLHQDWLNGKEYKCKVSNKALPAPIEKTISKAKGQPREPQVCTLPPSREEMTKNQVSLSCAVKGFYPSDIAVEWESNGQPENNYKTTPPVLDSDGSFFLVSKLTVDKSRWQQGNVFSCSVMHEALHNHYTQKSLSLSPGK

SEQ ID NO: 102 - protein, 458 aa, Artificial Sequence
  CHAIN: Sequence of BU4 chain 3 (BU4-H2)
QVQLQQSGAEVKKPGSSVRVSCKASGGTFNNNAINWVRQAPGQGLEWMGGIIPMFGTAKYSQNFQGRVAITADESTGTASMELSSLRSEDTAVYYCARSRDLLLFPHHALSPWGRGTMVTVSSGGGGSKAGIRGIPPKIECLPSDISIDEGKVLTVASAFTGEPTPEVTWSTGGRKIHSQEQGRFHIESTEDLTTLIISDVQKQDGGLYSLSLGNEFGSDSATVNIHIRSIDKTHTCPPCPAPEAAGGPSVFLFPPKPKDTLMISRTPEVTCVVVDVSHEDPEVKFNWYVDGVEVHNAKTKPREEQYNSTYRVVSVLTVLHQDWLNGKEYKCKVSNKALPAPIEKTISKAKGQPREPQVCTLPPSREEMTKNQVSLSCAVKGFYPSDIAVEWESNGQPENNYKTTPPVLDSDGSFFLVSKLTVDKSRWQQGNVFSCSVMHEALHNHYTQKSLSLSPGK

SEQ ID NO: 103 - protein, 453 aa, Artificial Sequence
  CHAIN: Sequence of BU5 chain 1 (BU5-H1)
QVQLQQSGAEVKKPGSSVRVSCKASGGTFNNNAINWVRQAPGQGLEWMGGIIPMFGTAKYSQNFQGRVAITADESTGTASMELSSLRSEDTAVYYCARSRDLLLFPHHALSPWGRGTMVTVSSGGGGSGIPPKIECLPIDISIDEGKVLTVASAFTGEPTPEVTWSTGGRKIHSQEQGRFHIENTDDLTTLIIKDVQKQDGGLYTLTLRNEFGSDSATVNIHIRSIDKTHTCPPCPAPEAAGGPSVFLFPPKPKDTLMISRTPEVTCVVVDVSHEDPEVKFNWYVDGVEVHNAKTKPREEQYNSTYRVVSVLTVLHQDWLNGKEYKCKVSNKALPAPIEKTISKAKGQPREPQVCTLPPSREEMTKNQVSLSCAVKGFYPSDIAVEWESNGQPENNYKTTPPVLDSDGSFFLVSKLTVDKSRWQQGNVFSCSVMHEALHNHYTQKSLSLSPGK

SEQ ID NO: 104 - protein, 210 aa, Artificial Sequence
  CHAIN: Sequence of BU5 chain 2 (BU5-L1)
SSELTQDPAVSVALGQTVRVTCQGDSLRSYYASWYQQKPGQAPVLVIYGKNNRPSGIPDRFSGSSSGNTASLTITGAQAEDEADYYCSSRDSSGNHWVFGGGTELTVLGGGGSSGAPRFLTRPLAFVVSVGKDATLSSQIVGNPTPQVSWEKDKQPVTAGARFRLAQDGDLYRLKILDLQLSDSGQYVSRARNAIGEAFACLGLQVDAEA

SEQ ID NO: 105 - protein, 125 aa, Artificial Sequence
  DOMAIN: VH sequence of A0 antibody
EVQLVESGGGLVQPGGSLKLSCAASGFTFNKYAMNWVRQAPGKGLEWVARIRSKYNNYATYYADSVKDRFTISRDDSKNTAYLQMNNLKTEDTAVYYCVRHGNFGNEYISYWAYWGQGTLVTVSS

SEQ ID NO: 106 - protein, 109 aa, Artificial Sequence
  DOMAIN: VL sequence of A0 antibody
QTVVTQEPSLTVSPGGTVTLTCGSSTGAVTSGNYPNWVQQKPGQAPRGLIGGTKFLAPGTPARFSGSLLGGKAALTLSGVQPEDEAEYYCVLWYSNRWVFGGGTKLTVL

SEQ ID NO: 107 - protein, 449 aa, Artificial Sequence
  CHAIN: Sequence of FA-1 chain 1 (FA-1-H1)
QVQLVQSGGGVVQPGTSLRLSCAASGFIFSSSAMHWVRQAPGKGLEWVAVISYDGSNKYYVDSVKGRFTISRDNSKNTLYLQMNSLRAEDTAVYYCARSARLYASFDYWGQGALVTVSSGGGGSGIPPKIECLPIDISIDEGKVLTVASAFTGEPTPEVTWSTGGRKIHSQEQGRFHIENTDDLTTLIIKDVQKQDGGLYTLTLRNEFGSDSATVNIHIRSIDKTHTCPPCPAPEAAGGPSVFLFPPKPKDTLMISRTPEVTCVVVDVSHEDPEVKFNWYVDGVEVHNAKTKPREEQYNSTYRVVSVLTVLHQDWLNGKEYKCKVSNKALPAPIEKTISKAKGQPREPQVCTLPPSREEMTKNQVSLSCAVKGFYPSDIAVEWESNGQPENNYKTTPPVLDSDGSFFLVSKLTVDKSRWQQGNVFSCSVMHEALHNHYTQKSLSLSPGK

SEQ ID NO: 108 - protein, 212 aa, Artificial Sequence
  CHAIN: Sequence of FA-1 chain 2 (FA-1-L1)
DTVVTQEPSFSVSPGGTVTLTCGLSSGSVSTSHYPSWYQQTPGQAPRMLIYNTNTRSSGVPDRFSGSILGNKAALTITGAQADDESDYYCAIHVDRDIWVFGGGTKLTVLGGGGSSGAPRFLTRPLAFVVSVGKDATLSSQIVGNPTPQVSWEKDKQPVTAGARFRLAQDGDLYRLKILDLQLSDSGQYVSRARNAIGEAFACLGLQVDAEA

SEQ ID NO: 109 - protein, 455 aa, Artificial Sequence
  CHAIN: Sequence of FA-1 chain 3 (FA-1-H2)
EVQLVESGGGLVQPGGSLKLSCAASGFTFNKYAMNWVRQAPGKGLEWVARIRSKYNNYATYYADSVKDRFTISRDDSKNTAYLQMNNLKTEDTAVYYCVRHGNFGNEYISYWAYWGQGTLVTVSSASTKGPSVFPLAPSSKSTSGGTAALGCLVKDYFPEPVTVSWNSGALTSGVHTFPAVLQSSGLYSLSSVVTVPSSSLGTQTYICNVNHKPSNTKVDKKVEPKSCDKTHTCPPCPAPEAAGGPSVFLFPPKPKDTLMISRTPEVTCVVVDVSHEDPEVKFNWYVDGVEVHNAKTKPREEQYNSTYRVVSVLTVLHQDWLNGKEYKCKVSNKALPAPIEKTISKAKGQPREPQVYTLPPCREEMTKNQVSLWCLVKGFYPSDIAVEWESNGQPENNYKTTPPVLDSDGSFFLYSKLTVDKSRWQQGNVFSCSVMHEALHNHYTQKSLSLSPGK

SEQ ID NO: 110 - protein, 216 aa, Artificial Sequence
  CHAIN: Sequence of FA-1 chain 4 (FA-1-L2)
QTVVTQEPSLTVSPGGTVTLTCGSSTGAVTSGNYPNWVQQKPGQAPRGLIGGTKFLAPGTPARFSGSLLGGKAALTLSGVQPEDEAEYYCVLWYSNRWVFGGGTKLTVLRTVAAPSVFIFPPSDEQLKSGTASVVCLLNNFYPREAKVQWKVDNALQSGNSQESVTEQDSKDSTYSLSSTLTLSKADYEKHKVYACEVTHQGLSSPVTKSFNRGEC

SEQ ID NO: 111 - protein, 447 aa, Artificial Sequence
  DOMAIN: Sequence of hB7H3 antigen protein
LEVQVPEDPVVALVGTDATLCCSFSPEPGFSLAQLNLIWQLTDTKQLVHSFAEGQDQGSAYANRTALFPDLLAQGNASLRLQRVRVADEGSFTCFVSIRDFGSAAVSLQVAAPYSKPSMTLEPNKDLRPGDTVTITCSSYQGYPEAEVFWQDGQGVPLTGNVTTSQMANEQGLFDVHSILRVVLGANGTYSCLVRNPVLQQDAHSSVTITPQRSPTGAVEVQVPEDPVVALVGTDATLRCSFSPEPGFSLAQLNLIWQLTDTKQLVHSFTEGRDQGSAYANRTALFPDLLAQGNASLRLQRVRVADEGSFTCFVSIRDFGSAAVSLQVAAPYSKPSMTLEPNKDLRPGDTVTITCSSYRGYPEAEVFWQDGQGVPLTGNVTTSQMANEQGLFDVHSVLRVVLGANGTYSCLVRNPVLQQDAHGSVTITGQPMTDYKDDDDKHHHHHH

SEQ ID NO: 112 - protein, 126 aa, Artificial Sequence
  DOMAIN: Sequence of delta subunit of hCD3 antigen
FKIPIEELEDRVFVNCNTSITWVEGTVGTLLSDITRLDLGKRILDPRGIYRCNGTDIYKDKESTVQVHYRMCQSCVELDPATVASAENAQCEKELQALEKENAQLEWELQALEKELAQDYKDDDDK

SEQ ID NO: 113 - protein, 143 aa, Artificial Sequence
  DOMAIN: Sequence of epsilon subunit of hCD3 antigen
DGNEEMGGITQTPYKVSISGTTVILTCPQYPGSEILWQHNDKNIGGDEDDKNIGSDEDHLSLKEFSELEQSGYYVCYPRGSKPEDANFYLYLRARVCENCMEMDAKNAQCKKKLQALKKKNAQLKWKLQALKKKLAQHHHHHH

SEQ ID NO: 114 - protein, 482 aa, Artificial Sequence
  CHAIN: Sequence of HJ-1-H1
EVQLVESGGGLVQPGGSLRLSCAASGFTFSHYYMAWVRQAPGKGLEWVTSISYEGDITYYGDSVKGRFTISRDNSKNTLYLQMNSLRAEDTATYYCASQTLRESFDYWGQGTLVTVSSLEDLKNVFPPEVAVFEPSEAEISHTQKATLVCLATGFYPDHVELSWWVNGKEVHSGVCTDPQPLKEQPALQDSRYALSSRLRVSATFWQNPRNHFRCQVQFYGLSENDEWTQDRAKPVTQIVSAEAWGRASDKTHTCPPCPAPEAAGGPSVFLFPPKPKDTLMISRTPEVTCVVVDVSHEDPEVKFNWYVDGVEVHNAKTKPREEQYNSTYRVVSVLTVLHQDWLNGKEYKCKVSNKALPAPIEKTISKAKGQPREPQVYTLPPCREEMTKNQVSLWCLVKGFYPSDIAVEWESNGQPENNYKTTPPVLDSDGSFFLYSKLTVDKSRWQQGNVFSCSVMHEALHNHYTQKSLSLSPGKHHHHHH

SEQ ID NO: 115 - protein, 203 aa, Artificial Sequence
  CHAIN: Sequence of HJ-1-L1
DIQMTQSPSSVSASVGDRVTITCRASQDIANYLSWYQQKPGKSPKLLIYGTSNLEVGVPSRFSGSRSGTDFTLTISSLQPEDFATYYCLQDKEFPRTFGGGTKVEIKKPDIQNPDPAVYQLRDSKSSDKSVCLFTDFDSQTQVSQSKDSDVYITDKCVLDMRSMDFKSNSAVAWSQKSDFACANAFQNSIIPEDTFFPSPESS

SEQ ID NO: 116 - protein, 457 aa, Artificial Sequence
  CHAIN: Sequence of HJ-1-H2/HJ-3-H2
EVQLVQSGAEVKKPGSSVKVSCKASGYTFSNYLIEWVRQAPGQGLEWIGVIDPGVGDTNYNENFKGRATLTADKSTSTAYIELSSLRSEDTAVYYCAREDNTGTAFDYWGQGTTVTVSSASTKGPSVFPLAPSSKSTSGGTAALGCLVKDYFPEPVTVSWNSGALTSGVHTFPAVLQSSGLYSLSSVVTVPSSSLGTQTYICNVNHKPSNTKVDKKVEPKSCDKTHTCPPCPAPEAAGGPSVFLFPPKPKDTLMISRTPEVTCVVVDVSHEDPEVKFNWYVDGVEVHNAKTKPREEQYNSTYRVVSVLTVLHQDWLNGKEYKCKVSNKALPAPIEKTISKAKGQPREPQVCTLPPSREEMTKNQVSLSCAVKGFYPSDIAVEWESNGQPENNYKTTPPVLDSDGSFFLVSKLTVDKSRWQQGNVFSCSVMHEALHNHYTQKSLSLSPGKDYKDDDDK

SEQ ID NO: 117 - protein, 214 aa, Artificial Sequence
  CHAIN: Sequence of HJ-1-L2/HJ-3-L2
SIVMTQTPLSLSVTPGQPASISCKASQSVSSDVTWYLQKPGQSPQLLIYYVSEHYTGVPDRFSGSGYGTDFTLKISRVEAEDVGVYYCQQHHRFPLTFGQGTKLEIKRTVAAPSVFIFPPSDEQLKSGTASVVCLLNNFYPREAKVQWKVDNALQSGNSQESVTEQDSKDSTYSLSSTLTLSKADYEKHKVYACEVTHQGLSSPVTKSFNRGEC

SEQ ID NO: 118 - protein, 456 aa, Artificial Sequence
  CHAIN: Sequence of HJ-2-H1/HJ-4-H1
EVQLVESGGGLVQPGGSLRLSCAASGFTFSHYYMAWVRQAPGKGLEWVTSISYEGDITYYGDSVKGRFTISRDNSKNTLYLQMNSLRAEDTATYYCASQTLRESFDYWGQGTLVTVSSASTKGPSVFPLAPSSKSTSGGTAALGCLVKDYFPEPVTVSWNSGALTSGVHTFPAVLQSSGLYSLSSVVTVPSSSLGTQTYICNVNHKPSNTKVDKKVEPKSCDKTHTCPPCPAPEAAGGPSVFLFPPKPKDTLMISRTPEVTCVVVDVSHEDPEVKFNWYVDGVEVHNAKTKPREEQYNSTYRVVSVLTVLHQDWLNGKEYKCKVSNKALPAPIEKTISKAKGQPREPQVCTLPPSREEMTKNQVSLSCAVKGFYPSDIAVEWESNGQPENNYKTTPPVLDSDGSFFLVSKLTVDKSRWQQGNVFSCSVMHEALHNHYTQKSLSLSPGKDYKDDDDK

SEQ ID NO: 119 - protein, 214 aa, Artificial Sequence
  CHAIN: Sequence of HJ-2-L1/HJ-4-L1
DIQMTQSPSSVSASVGDRVTITCRASQDIANYLSWYQQKPGKSPKLLIYGTSNLEVGVPSRFSGSRSGTDFTLTISSLQPEDFATYYCLQDKEFPRTFGGGTKVEIKRTVAAPSVFIFPPSDEQLKSGTASVVCLLNNFYPREAKVQWKVDNALQSGNSQESVTEQDSKDSTYSLSSTLTLSKADYEKHKVYACEVTHQGLSSPVTKSFNRGEC

SEQ ID NO: 120 - protein, 483 aa, Artificial Sequence
  CHAIN: Sequence of HJ-1-H2
EVQLVQSGAEVKKPGSSVKVSCKASGYTFSNYLIEWVRQAPGQGLEWIGVIDPGVGDTNYNENFKGRATLTADKSTSTAYIELSSLRSEDTAVYYCAREDNTGTAFDYWGQGTTVTVSSLEDLKNVFPPEVAVFEPSEAEISHTQKATLVCLATGFYPDHVELSWWVNGKEVHSGVCTDPQPLKEQPALQDSRYALSSRLRVSATFWQNPRNHFRCQVQFYGLSENDEWTQDRAKPVTQIVSAEAWGRASDKTHTCPPCPAPEAAGGPSVFLFPPKPKDTLMISRTPEVTCVVVDVSHEDPEVKFNWYVDGVEVHNAKTKPREEQYNSTYRVVSVLTVLHQDWLNGKEYKCKVSNKALPAPIEKTISKAKGQPREPQVYTLPPCREEMTKNQVSLWCLVKGFYPSDIAVEWESNGQPENNYKTTPPVLDSDGSFFLYSKLTVDKSRWQQGNVFSCSVMHEALHNHYTQKSLSLSPGKHHHHHH

SEQ ID NO: 121 - protein, 203 aa, Artificial Sequence
  CHAIN: Sequence of HJ-2-L2
SIVMTQTPLSLSVTPGQPASISCKASQSVSSDVTWYLQKPGQSPQLLIYYVSEHYTGVPDRFSGSGYGTDFTLKISRVEAEDVGVYYCQQHHRFPLTFGQGTKLEIKKPDIQNPDPAVYQLRDSKSSDKSVCLFTDFDSQTQVSQSKDSDVYITDKCVLDMRSMDFKSNSAVAWSQKSDFACANAFQNSIIPEDTFFPSPESS

SEQ ID NO: 122 - protein, 454 aa, Artificial Sequence
  CHAIN: Sequence of HJ-3-H1
EVQLVESGGGLVQPGGSLRLSCAASGFTFSHYYMAWVRQAPGKGLEWVTSISYEGDITYYGDSVKGRFTISRDNSKNTLYLQMNSLRAEDTATYYCASQTLRESFDYWGQGTLVTVSSGGGGSGIPPKIECLPIDISIDEGKVLTVASAFTGEPTPEVTWSTGGRKIHSQEQGRFHIENTDDLTTLIIKDVQKQDGGLYTLTLRNEFGSDSATVNIHIRSIDKTHTCPPCPAPEAAGGPSVFLFPPKPKDTLMISRTPEVTCVVVDVSHEDPEVKFNWYVDGVEVHNAKTKPREEQYNSTYRVVSVLTVLHQDWLNGKEYKCKVSNKALPAPIEKTISKAKGQPREPQVYTLPPCREEMTKNQVSLWCLVKGFYPSDIAVEWESNGQPENNYKTTPPVLDSDGSFFLYSKLTVDKSRWQQGNVFSCSVMHEALHNHYTQKSLSLSPGKHHHHHH

SEQ ID NO: 123 - protein, 209 aa, Artificial Sequence
  CHAIN: Sequence of HJ-3-L1
DIQMTQSPSSVSASVGDRVTITCRASQDIANYLSWYQQKPGKSPKLLIYGTSNLEVGVPSRFSGSRSGTDFTLTISSLQPEDFATYYCLQDKEFPRTFGGGTKVEIKGGGGSSGAPRFLTRPLAFVVSVGKDATLSSQIVGNPTPQVSWEKDKQPVTAGARFRLAQDGDLYRLKILDLQLSDSGQYVSRARNAIGEAFACLGLQVDAEA

SEQ ID NO: 124 - protein, 455 aa, Artificial Sequence
  CHAIN: Sequence of HJ-4-H2
EVQLVQSGAEVKKPGSSVKVSCKASGYTFSNYLIEWVRQAPGQGLEWIGVIDPGVGDTNYNENFKGRATLTADKSTSTAYIELSSLRSEDTAVYYCAREDNTGTAFDYWGQGTTVTVSSGGGGSGIPPKIECLPIDISIDEGKVLTVASAFTGEPTPEVTWSTGGRKIHSQEQGRFHIENTDDLTTLIIKDVQKQDGGLYTLTLRNEFGSDSATVNIHIRSIDKTHTCPPCPAPEAAGGPSVFLFPPKPKDTLMISRTPEVTCVVVDVSHEDPEVKFNWYVDGVEVHNAKTKPREEQYNSTYRVVSVLTVLHQDWLNGKEYKCKVSNKALPAPIEKTISKAKGQPREPQVYTLPPCREEMTKNQVSLWCLVKGFYPSDIAVEWESNGQPENNYKTTPPVLDSDGSFFLYSKLTVDKSRWQQGNVFSCSVMHEALHNHYTQKSLSLSPGKHHHHHH

SEQ ID NO: 125 - protein, 209 aa, Artificial Sequence
  CHAIN: Sequence of HJ-4-L2
SIVMTQTPLSLSVTPGQPASISCKASQSVSSDVTWYLQKPGQSPQLLIYYVSEHYTGVPDRFSGSGYGTDFTLKISRVEAEDVGVYYCQQHHRFPLTFGQGTKLEIKGGGGSSGAPRFLTRPLAFVVSVGKDATLSSQIVGNPTPQVSWEKDKQPVTAGARFRLAQDGDLYRLKILDLQLSDSGQYVSRARNAIGEAFACLGLQVDAEA

SEQ ID NO: 126 - protein, 449 aa, Artificial Sequence
  CHAIN: Heavy chain sequence of J1
EVQLVQSGAEVKKPGSSVKVSCKASGYTFSNYLIEWVRQAPGQGLEWIGVIDPGVGDTNYNENFKGRATLTADKSTSTAYIELSSLRSEDTAVYYCAREDNTGTAFDYWGQGTTVTVSSASTKGPSVFPLAPSSKSTSGGTAALGCLVKDYFPEPVTVSWNSGALTSGVHTFPAVLQSSGLYSLSSVVTVPSSSLGTQTYICNVNHKPSNTKVDKKVEPKSCDKTHTCPPCPAPELLGGPSVFLFPPKPKDTLYITREPEVTCVVVDVSHEDPEVKFNWYVDGVEVHNAKTKPREEQYNSTYRVVSVLTVLHQDWLNGKEYKCKVSNKALPAPIEKTISKAKGQPREPQVYTLPPSRDELTKNQVSLTCLVKGFYPSDIAVEWESNGQPENNYKTTPPVLDSDGSFFLYSKLTVDKSRWQQGNVFSCSVMHEALHNHYTQKSLSLSPGK

SEQ ID NO: 127 - protein, 103 aa, Artificial Sequence
  DOMAIN: T.6 chain sequence
KAGIRGIPPKIEALPSDISIDEGKVLTVACAFTGEPTPEVTWSCGGRKIHSQEQGRFHIENTDDLTTLIIMDVQKQDGGLYTLSLGNEFGSDSATVNIHIRSI

SEQ ID NO: 128 - protein, 102 aa, Artificial Sequence
  DOMAIN: O.16 chain sequence
DQPQFSGAPRFLTRPKAFVVSVGKDATLSCQIVGNPTPQVSWEKDQQPVAAGARFRLAQDGDLYRLTILDLALGDSGQYVCRARNAIGEAFAAVGLQVDAEA

SEQ ID NO: 129 - protein, 98 aa, Artificial Sequence
  DOMAIN: T.16 chain sequence
GIPPKIECLPIDISIDEGKVLTVASAFTGEPTPEVTWSTGGRKIHSQEQGRFHIENTDDSTTLTIKDVQKQDGGLYTLTLRNEFGSDSATVNIHIRSI

SEQ ID NO: 130 - protein, 98 aa, Artificial Sequence
  DOMAIN: T.17 chain sequence
GIPPKIECLPIDISIDEGKCLTVASAFTGEPTPEVTWSTGGRKIHSQEQGRFHIENTDDSTTLTIKDVQKQDGGLYTLTLRNEFGSDSATVNIHIRSI

SEQ ID NO: 131 - protein, 98 aa, Artificial Sequence
  DOMAIN: T.18 chain sequence
GIPPKIECLPIDISIDEGKVLTVASCFTGEPTPEVTWSTGGRKIHSQEQGRFHIENTDDSTTLTIKDVQKQDGGLYTLTLRNEFGSDSATVNIHIRSI

SEQ ID NO: 132 - protein, 97 aa, Artificial Sequence
  DOMAIN: O.24 chain sequence
SGAPRFLTRPKAFVVSVGKDATLSSQIVGNPFPQVSWEKDKQPVTAGVRFRLAQDGDLYRLKILDLQLSDSGQYVSRARNAIGEAFACLGLQVDAEA

SEQ ID NO: 133 - protein, 97 aa, Artificial Sequence
  DOMAIN: O.25 chain sequence
SGAPRFLTRPKASVVSVGKDATLSSQIVGNPFPQVSWEKDKQPVTAGVRFRLAQDGDLYRLKILDLQLSDSGQYVSRARNAHGEAFACLGLQVDAEA

SEQ ID NO: 134 - protein, 97 aa, Artificial Sequence
  DOMAIN: O.26 chain sequence
SGCPRFLTRPKASVVSVGKDATLSSQIVGNPFPQVSWEKDKQPVTAGVRFRLAQDGDLYRLKILDLQLSDSGQYVSRARNAHGEAFACLGLQVDAEA

SEQ ID NO: 135 - protein, 97 aa, Artificial Sequence
  DOMAIN: O.27 chain sequence
SGAPRFLTCPKASVVSVGKDATLSSQIVGNPFPQVSWEKDKQPVTAGVRFRLAQDGDLYRLKILDLQLSDSGQYVSRARNAHGEAFACLGLQVDAEA

SEQ ID NO: 136 - protein, 97 aa, Artificial Sequence
  DOMAIN: O.28 chain sequence
SGAPRFLTRPKASVVSVGKDATLSCQIVGNPFPQVSWEKDKQPVTAGVRFRLAQDGDLYRLKILDLQLSDSGQYVCRARNAHGEAFACLGLQVDAEA

SEQ ID NO: 137 - protein, 97 aa, Artificial Sequence
  DOMAIN: O.29 chain sequence
SGCPRFLTRPKASVVSVGKDATLSCQIVGNPFPQVSWEKDKQPVTAGVRFRLAQDGDLYRLKILDLQLSDSGQYVCRARNAHGEAFACLGLQVDAEA

SEQ ID NO: 138 - protein, 97 aa, Artificial Sequence
  DOMAIN: O.30 chain sequence
SGAPRFLTCPKASVVSVGKDATLSCQIVGNPFPQVSWEKDKQPVTAGVRFRLAQDGDLYRLKILDLQLSDSGQYVCRARNAHGEAFACLGLQVDAEA

SEQ ID NO: 139 - protein, 97 aa, Artificial Sequence
  DOMAIN: O.31 chain sequence
SGAPRFLTRPKASVVSVGKDATLSSQIVGNPFPQVSWEKDKQPVTAGVRFRLAQDGDLYRLKILDCQLSDSGQYVSRARNAHGEAFACLGLQCDAEA

SEQ ID NO: 140 - protein, 97 aa, Artificial Sequence
  DOMAIN: O.32 chain sequence
SGCPRFLTRPKASVVSVGKDATLSSQIVGNPFPQVSWEKDKQPVTAGVRFRLAQDGDLYRLKILDCQLSDSGQYVSRARNAHGEAFACLGLQCDAEA

SEQ ID NO: 141 - protein, 97 aa, Artificial Sequence
  DOMAIN: O.33 chain sequence
SGAPRFLTCPKASVVSVGKDATLSSQIVGNPFPQVSWEKDKQPVTAGVRFRLAQDGDLYRLKILDCQLSDSGQYVSRARNAHGEAFACLGLQCDAEA

SEQ ID NO: 142 - protein, 448 aa, Artificial Sequence
  CHAIN: First heavy chain sequence of PL-1
QVQLVQSGAEVKKPGASVKVSCKASGYTFTSYWMHWVRQAPGQGLEWMGRITPSSGFAMYNEKFKNRVTMTRDTSTSTVYMELSSLRSEDTAVYYCARGGSSYDYFDYWGQGTTVTVSSGGGGSSGAPRFLTRPLAFVVSVGKDATLSSQIVGNPTPQVSWEKDKQPVTAGARFRLAQDGDLYRLKILDLQLSDSGQYVSRARNAIGEAFACLGLQVDAEADKTHTCPPCPAPEAAGGPSVFLFPPKPKDTLMISRTPEVTCVVVDVSHEDPEVKFNWYVDGVEVHNAKTKPREEQYNSTYRVVSVLTVLHQDWLNGKEYKCKVSNKALPAPIEKTISKAKGQPREPQVYTLPPCREEMTKNQVSLWCLVKGFYPSDIAVEWESNGQPENNYKTTPPVLDSDGSFFLYSKLTVDKSRWQQGNVFSCSVMHEALHNHYTQKSLSLSPGK

SEQ ID NO: 143 - protein, 214 aa, Artificial Sequence
  CHAIN: First light chain sequence of PL-1
DIVLTQSPASLAVSPGQRATITCRASESVSIHGTHLMHWYQQKPGQPPKLLIYAASKLESGVPARFSGSGSGTDFTLTINPVEAEDTANYYCQQSFEDPLTFGQGTKLEIKGGGGSGIPPKIECLPIDISIDEGKVLTVASAFTGEPTPEVTWSTGGRKIHSQEQGRFHIENTDDLTTLIIKDVQKQDGGLYTLTLRNEFGSDSATVNIHIRSI

SEQ ID NO: 144 - protein, 448 aa, Artificial Sequence
  CHAIN: Second heavy chain sequence of PL-1
QVQLVESGGGVVQPGRSLRLSCAASGFTFSSYTMHWVRQAPGKGLEWVTFISYDGNNKYYADSVKGRFTISRDNSKNTLYLQMNSLRAEDTAIYYCARTGWLGPFDYWGQGTLVTVSSASTKGPSVFPLAPSSKSTSGGTAALGCLVKDYFPEPVTVSWNSGALTSGVHTFPAVLQSSGLYSLSSVVTVPSSSLGTQTYICNVNHKPSNTKVDKKVEPKSCDKTHTCPPCPAPEAAGGPSVFLFPPKPKDTLMISRTPEVTCVVVDVSHEDPEVKFNWYVDGVEVHNAKTKPREEQYNSTYRVVSVLTVLHQDWLNGKEYKCKVSNKALPAPIEKTISKAKGQPREPQVCTLPPSREEMTKNQVSLSCAVKGFYPSDIAVEWESNGQPENNYKTTPPVLDSDGSFFLVSKLTVDKSRWQQGNVFSCSVMHEALHNHYTQKSLSLSPGK

SEQ ID NO: 145 - protein, 215 aa, Artificial Sequence
  CHAIN: Second light chain sequence of PL-1
EIVLTQSPGTLSLSPGERATLSCRASQSVGSSYLAWYQQKPGQAPRLLIYGAFSRATGIPDRFSGSGSGTDFTLTISRLEPEDFAVYYCQQYGSSPWTFGQGTKVEIKRTVAAPSVFIFPPSDEQLKSGTASVVCLLNNFYPREAKVQWKVDNALQSGNSQESVTEQDSKDSTYSLSSTLTLSKADYEKHKVYACEVTHQGLSSPVTKSFNRGEC

SEQ ID NO: 146 - protein, 214 aa, Artificial Sequence; identical to SEQ ID NO: 143
  CHAIN: Light chain 1 sequence of P-O-T

SEQ ID NO: 147 - protein, 214 aa, Artificial Sequence
  CHAIN: Light chain 2 sequence of P-O-T
DIQMTQSPSSLSASVGDRVTITCRASENIYSYLAWYQQKPGKSPKLLIYNARTLAEGVPSRFSGSGSGTDFTLTISSLQPEDFATYYCQYHSGSPLPFGGGTKVEIKRTVAAPSVFIFPPSDEQLKSGTASVVCLLNNFYPREAKVQWKVDNALQSGNSQESVTEQDSKDSTYSLSSTLTLSKADYEKHKVYACEVTHQGLSSPVTKSFNRGEC

SEQ ID NO: 148 - protein, 675 aa, Artificial Sequence
  CHAIN: Heavy chain sequence of P-O-T
QVQLVQSGAEVKKPGASVKVSCKASGYTFTSYWMHWVRQAPGQGLEWMGRITPSSGFAMYNEKFKNRVTMTRDTSTSTVYMELSSLRSEDTAVYYCARGGSSYDYFDYWGQGTTVTVSSGGGGSSGAPRFLTRPKAFVVSVGKDATLSSQIVGNPFPQVSWEKDKQPVTAGVRFRLAQDGDLYRLKILDLQLSDSGQYVSRARNAIGEAFACLGLQVDAEAGGGGSEVQLVQSGAEVKKPGASVKVSCKASGYTFTNYWMHWVRQAPGQGLEWMGRIDPDSTGSKYNEKFKTRVTMTRDTSTSTVYMELSSLRSEDTAVYYCAREGAYGYYFDYWGQGTLVTVSSASTKGPSVFPLAPSSKSTSGGTAALGCLVKDYFPEPVTVSWNSGALTSGVHTFPAVLQSSGLYSLSSVVTVPSSSLGTQTYICNVNHKPSNTKVDKKVEPKSCDKTHTCPPCPAPELLGGPSVFLFPPKPKDTLMISRTPEVTCVVVDVSHEDPEVKFNWYVDGVEVHNAKTKPREEQYNSTYRVVSVLTVLHQDWLNGKEYKCKVSNKALPAPIEKTISKAKGQPREPQVYTLPPSRDELTKNQVSLTCLVKGFYPSDIAVEWESNGQPENNYKTTPPVLDSDGSFFLYSKLTVDKSRWQQGNVFSCSVMHEALHNHYTQKSLSLSPGK

SEQ ID NO: 149 - protein, 214 aa, Artificial Sequence; identical to SEQ ID NO: 147
  CHAIN: Light chain sequence of h1708-04

SEQ ID NO: 150 - protein, 449 aa, Artificial Sequence
  CHAIN: Heavy chain sequence of h1708-04
EVQLVQSGAEVKKPGASVKVSCKASGYTFTNYWMHWVRQAPGQGLEWMGRIDPDSTGSKYNEKFKTRVTMTRDTSTSTVYMELSSLRSEDTAVYYCAREGAYGYYFDYWGQGTLVTVSSASTKGPSVFPLAPSSKSTSGGTAALGCLVKDYFPEPVTVSWNSGALTSGVHTFPAVLQSSGLYSLSSVVTVPSSSLGTQTYICNVNHKPSNTKVDKKVEPKSCDKTHTCPPCPAPELLGGPSVFLFPPKPKDTLMISRTPEVTCVVVDVSHEDPEVKFNWYVDGVEVHNAKTKPREEQYNSTYRVVSVLTVLHQDWLNGKEYKCKVSNKALPAPIEKTISKAKGQPREPQVYTLPPSRDELTKNQVSLTCLVKGFYPSDIAVEWESNGQPENNYKTTPPVLDSDGSFFLYSKLTVDKSRWQQGNVFSCSVMHEALHNHYTQKSLSLSPGK

SEQ ID NO: 151 - protein, 218 aa, Artificial Sequence
  CHAIN: Light chain sequence of h1831K
DIVLTQSPASLAVSPGQRATITCRASESVSIHGTHLMHWYQQKPGQPPKLLIYAASKLESGVPARFSGSGSGTDFTLTINPVEAEDTANYYCQQSFEDPLTFGQGTKLEIKRTVAAPSVFIFPPSDEQLKSGTASVVCLLNNFYPREAKVQWKVDNALQSGNSQESVTEQDSKDSTYSLSSTLTLSKADYEKHKVYACEVTHQGLSSPVTKSFNRGEC

SEQ ID NO: 152 - protein, 449 aa, Artificial Sequence
  CHAIN: Heavy chain sequence of h1831K
QVQLVQSGAEVKKPGASVKVSCKASGYTFTSYWMHWVRQAPGQGLEWMGRITPSSGFAMYNEKFKNRVTMTRDTSTSTVYMELSSLRSEDTAVYYCARGGSSYDYFDYWGQGTTVTVSSASTKGPSVFPLAPSSKSTSGGTAALGCLVKDYFPEPVTVSWNSGALTSGVHTFPAVLQSSGLYSLSSVVTVPSSSLGTQTYICNVNHKPSNTKVDKKVEPKSCDKTHTCPPCPAPELLGGPSVFLFPPKPKDTLMISRTPEVTCVVVDVSHEDPEVKFNWYVDGVEVHNAKTKPREEQYNSTYRVVSVLTVLHQDWLNGKEYKCKVSNKALPAPIEKTISKAKGQPREPQVYTLPPSRDELTKNQVSLTCLVKGFYPSDIAVEWESNGQPENNYKTTPPVLDSDGSFFLYSKLTVDKSRWQQGNVFSCSVMHEALHNHYTQKSLSLSPGK

SEQ ID NO: 153 - protein, 107 aa, Artificial Sequence
  DOMAIN: Light chain variable region sequence of h1708-04
DIQMTQSPSSLSASVGDRVTITCRASENIYSYLAWYQQKPGKSPKLLIYNARTLAEGVPSRFSGSGSGTDFTLTISSLQPEDFATYYCQYHSGSPLPFGGGTKVEIK

SEQ ID NO: 154 - protein, 119 aa, Artificial Sequence
  DOMAIN: Heavy chain variable region sequence of h1708-04
EVQLVQSGAEVKKPGASVKVSCKASGYTFTNYWMHWVRQAPGQGLEWMGRIDPDSTGSKYNEKFKTRVTMTRDTSTSTVYMELSSLRSEDTAVYYCAREGAYGYYFDYWGQGTLVTVSS

SEQ ID NO: 155 - protein, 111 aa, Artificial Sequence
  DOMAIN: Light chain variable region sequence of h1831K
DIVLTQSPASLAVSPGQRATITCRASESVSIHGTHLMHWYQQKPGQPPKLLIYAASKLESGVPARFSGSGSGTDFTLTINPVEAEDTANYYCQQSFEDPLTFGQGTKLEIK

SEQ ID NO: 156 - protein, 119 aa, Artificial Sequence
  DOMAIN: Heavy chain variable region sequence of h1831K
QVQLVQSGAEVKKPGASVKVSCKASGYTFTSYWMHWVRQAPGQGLEWMGRITPSSGFAMYNEKFKNRVTMTRDTSTSTVYMELSSLRSEDTAVYYCARGGSSYDYFDYWGQGTTVTVSS

SEQ ID NO: 157 - protein, 5 aa, Artificial Sequence
  DOMAIN: HCDR1 sequence of h1708-04
NYWMH

SEQ ID NO: 158 - protein, 17 aa, Artificial Sequence
  DOMAIN: HCDR2 sequence of h1708-04
RIDPDSTGSKYNEKFKT

SEQ ID NO: 159 - protein, 10 aa, Artificial Sequence
  DOMAIN: HCDR3 sequence of h1708-04
EGAYGYYFDY

SEQ ID NO: 160 - protein, 11 aa, Artificial Sequence
  DOMAIN: LCDR1 sequence of h1708-04
RASENIYSYLA

SEQ ID NO: 161 - protein, 7 aa, Artificial Sequence
  DOMAIN: LCDR2 sequence of h1708-04
NARTLAE

SEQ ID NO: 162 - protein, 9 aa, Artificial Sequence
  DOMAIN: LCDR3 sequence of h1708-04
QYHSGSPLP

SEQ ID NO: 163 - protein, 5 aa, Artificial Sequence
  DOMAIN: HCDR1 sequence of h1831K
SYWMH

SEQ ID NO: 164 - protein, 17 aa, Artificial Sequence
  DOMAIN: HCDR2 sequence of h1831K
RITPSSGFAMYNEKFKN

SEQ ID NO: 165 - protein, 10 aa, Artificial Sequence
  DOMAIN: HCDR3 sequence of h1831K
GGSSYDYFDY

SEQ ID NO: 166 - protein, 15 aa, Artificial Sequence
  DOMAIN: LCDR1 sequence of h1831K
RASESVSIHGTHLMH

SEQ ID NO: 167 - protein, 7 aa, Artificial Sequence
  DOMAIN: LCDR2 sequence of h1831K
AASKLES

SEQ ID NO: 168 - protein, 9 aa, Artificial Sequence
  DOMAIN: LCDR3 sequence of h1831K
QQSFEDPLT

SEQ ID NO: 169 - protein, 118 aa, Artificial Sequence
  DOMAIN: Heavy chain variable region sequence of L0
QVQLVESGGGVVQPGRSLRLSCAASGFTFSSYTMHWVRQAPGKGLEWVTFISYDGNNKYYADSVKGRFTISRDNSKNTLYLQMNSLRAEDTAIYYCARTGWLGPFDYWGQGTLVTVSS

SEQ ID NO: 170 - protein, 108 aa, Artificial Sequence
  DOMAIN: Light chain variable region sequence of L0
EIVLTQSPGTLSLSPGERATLSCRASQSVGSSYLAWYQQKPGQAPRLLIYGAFSRATGIPDRFSGSGSGTDFTLTISRLEPEDFAVYYCQQYGSSPWTFGQGTKVEIK

SEQ ID NO: 171 - protein, 119 aa, Artificial Sequence
  DOMAIN: Sequence of heavy chain variable region of J1
EVQLVQSGAEVKKPGSSVKVSCKASGYTFSNYLIEWVRQAPGQGLEWIGVIDPGVGDTNYNENFKGRATLTADKSTSTAYIELSSLRSEDTAVYYCAREDNTGTAFDYWGQGTTVTVSS

SEQ ID NO: 172 - protein, 107 aa, Artificial Sequence
  DOMAIN: Sequence of light chain variable region of J1
SIVMTQTPLSLSVTPGQPASISCKASQSVSSDVTWYLQKPGQSPQLLIYYVSEHYTGVPDRFSGSGYGTDFTLKISRVEAEDVGVYYCQQHHRFPLTFGQGTKLEIK

SEQ ID NO: 173 - protein, 5 aa, Artificial Sequence
  DOMAIN: Amino acid sequence of C-terminal truncated sequence 1 of CH1
ASTKG

SEQ ID NO: 174 - protein, 5 aa, Artificial Sequence
  DOMAIN: Amino acid sequence of C-terminal truncated sequence 1 of CL
RTVAS

SEQ ID NO: 175 - protein, 5 aa, Artificial Sequence
  DOMAIN: Amino acid sequence of linker sequence 1
GGGGS

SEQ ID NO: 176 - protein, 10 aa, Artificial Sequence
  DOMAIN: Amino acid sequence of linker sequence 2
GGGGSGGGGS

SEQ ID NO: 177 - protein, 227 aa, Artificial Sequence
  DOMAIN: Sequence of Fc portion of heavy chain constant region of hole-IgG1
DKTHTCPPCPAPEAAGGPSVFLFPPKPKDTLMISRTPEVTCVVVDVSHEDPEVKFNWYVDGVEVHNAKTKPREEQYNSTYRVVSVLTVLHQDWLNGKEYKCKVSNKALPAPIEKTISKAKGQPREPQVCTLPPSREEMTKNQVSLSCAVKGFYPSDIAVEWESNGQPENNYKTTPPVLDSDGSFFLVSKLTVDKSRWQQGNVFSCSVMHEALHNHYTQKSLSLSPGK

SEQ ID NO: 178 - protein, 227 aa, Artificial Sequence
  DOMAIN: Sequence of Fc portion of heavy chain constant region of knob-IgG1
DKTHTCPPCPAPEAAGGPSVFLFPPKPKDTLMISRTPEVTCVVVDVSHEDPEVKFNWYVDGVEVHNAKTKPREEQYNSTYRVVSVLTVLHQDWLNGKEYKCKVSNKALPAPIEKTISKAKGQPREPQVYTLPPCREEMTKNQVSLWCLVKGFYPSDIAVEWESNGQPENNYKTTPPVLDSDGSFFLYSKLTVDKSRWQQGNVFSCSVMHEALHNHYTQKSLSLSPGK

SEQ ID NO: 179 - protein, 103 aa, Artificial Sequence
  DOMAIN: Sequence of CH1 portion of heavy chain constant region of IgG1
ASTKGPSVFPLAPSSKSTSGGTAALGCLVKDYFPEPVTVSWNSGALTSGVHTFPAVLQSSGLYSLSSVVTVPSSSLGTQTYICNVNHKPSNTKVDKKVEPKSC

SEQ ID NO: 180 - protein, 5 aa, Artificial Sequence
  Titin N-terminal 5AA
KAGIR

SEQ ID NO: 181 - protein, 5 aa, Artificial Sequence
  Obscurin N-terminal 5AA
DQPQF